European Patent Application EP 4 339 290 A1, published March 20, 2024. Title: USE OF PROTOPORPHYRINOGEN OXIDASE. Applicant: BEIJING DABEINONG BIOTECHNOLOGY CO., LTD. The sequence listing filed with the application follows.

SEQUENCE LISTING (81 sequences)

SEQ ID NO: 1 - protein, 179 aa, The amino acid sequence of PPO1(Ewingella americana)
MKALVLYSTRDGQTHAIASYIANCMKEKYECDVIDLLHAQHVTLSRYDKVLVGASIRYGHFNAVLDKFVKQNIQQLNSMPSAFFAVNLTARKPEKRTPQTNSYVRKFLLGTPWKPAMCGVFAGALRYPRYRWVDKVMIQLIMRMTGGETDTSKEVEYTDWEQVKKFAEDFGKLSYKKTL

SEQ ID NO: 2 - protein, 174 aa, The amino acid sequence of PPO2(Vibrio sp. HDW18)
MRALLLYSSQEGQTRKIIQRIAAQMPEYTCEVQDLHQSIDIDWAEYDKVLIGASIRYGRLNPALYRFIEHHLVGLTSRKAAFFCVNLTARKEQQGKDTPQGSAYIQTFLKKSAWQPERIAVFAGALYYPRYRWFDKMMIRLIMTLTGGETDTSQEVEYTNWDKVVKFAEQFRNW

SEQ ID NO: 3 - protein, 176 aa, The amino acid sequence of PPO3(Proteus hauseri)
MSALLLYCSTDGQTKKIMTQIANELRQHGYECDVRDLTSVQQNLNLSAYNKVLVGASIRYGYFNKALDKFITRHLSQLNNMPSAFFGVNLTARKEEKSTPETNSYICKFLDKTPWKPTLTGVFAGALFYPRYKWIDRVMIQLIMKMTKGETDPTKEIEYTDWNKVSEFATNFAKIG

SEQ ID NO: 4 - protein, 171 aa, The amino acid sequence of PPO4(Rodentibacter genomosp. 2)
MKTLILYSSHDGQTKKISEFLTALLNGEVLVDALREDYDIETFDQVIIGASIRYGHFSKTLDRFVVRNRVHLEQKRAVFFSVNLTARKEGKDNPETNVYVRKFLQRTKWQPKLAAVFAGALLYPRYKWFDRVMIRFIMKITGGETDITKEIEYTDWEKVREFAQRINRLEK

SEQ ID NO: 5 - protein, 176 aa, The amino acid sequence of PPO5(Mannheimia pernigra)
MKTLILYFTTDGQTKKIAERLADVITHEVELISLKDQAVDFAQKMANVDQVVIGASIRYGHFSPLVYQFIEQHYAMLNEKKTAFYGVNLTARKANRNTPTTNTYIRNFLAKVKWQPNYVEVIAGALFYPRYRFIDRMMIRFIMKVTKGETDVSKEYEYTNWQQVEEFGKKLSDQLI

SEQ ID NO: 6 - protein, 231 aa, The amino acid sequence of PPO6(Leptomonas pyrrhocoris)
MSSPNGKYLMLYSTTDGHTKTIMDTMAKHIMEEAKVQCDVVDMRDGDKYELAAYEKVMLGASIRYGFFSRTLHTYTTHHVDELNSMPSAFFGVNLTARKTSKNTAMTNAYTRKFLDQSMWVPQLSGVFAGALWYPRYNFFDRVMIQFIMKVTGGETNTTKEIVYTDWDAVHKFATDFVQLPATAIPRSKPATSVPPASVANYDNGARVALVVVGISAAIIFGRRLILAKRF

SEQ ID NO: 7 - protein, 174 aa, The amino acid sequence of PPO7(Aeromonas aquatica)
MDKILVLYSSQDGQTRKIVDAMLEEISGCDVVIQDLHTLPKCNLSKYAKVLIGASIRYGNFHPSLLSFINAHHEQLEVANAAFFCVNLTARKPEKQTPQTNAYMKKFLRLSPWKPKTLGVFAGALQYSRYNWWQTRIIQLIMKMTGGSTDTSQDLEFTDWVKVRSFAREFWSKR

SEQ ID NO: 8 - protein, 191 aa, The amino acid sequence of PPO8(Psychromonas sp. SA13A)
MSNETQAKQAETKQTESSVVSKTLVLYSSVDGQTLKIINRIKQTLTGEVIVLNVDDNPTIDFSLYQKVLIGASIRYGNFRPNIIKFVNQHKTQLDAVCNAFFVVCLTARKPEKAVPENNAYMKKFDQLSQWQPQFKGVFAGALLYSRYNWWQTLLIQLIMKMTGGSTDKTQDIELTDWEKVDSFAQDFAAR

SEQ ID NO: 9 - protein, 174 aa, The amino acid sequence of PPO9(Photobacterium aquae)
MEKVLLLHSSSDGQTVKILRHIETTLGGDYQCELVDLNTLPTVDFADYDRVLVGASIRYGHLNKKLYQFIERYRDELDQNKVGFFCVNLTARKEGKNTPETSVYMKTFLKKSPWCPKLQEVFAGALRYPRYGWFDRVMIQFIMRITGGETDTSKEVEYTDWQKVEAFAARFKHY

SEQ ID NO: 10 - protein, 174 aa, The amino acid sequence of PPO10(Vibrio mimicus)
MKALFLYSSQEGQTRKIIERIAQQMPEYDCDIQDLHQVSDIALADYDKILIGASIRYGRLNDKLYQFIQRYLPDLRSNKAAFFCVNLTARKEEQGKDTPEGSVYIQTFLKKSPWQPERIAVFAGALYYPRYRWFDKMMIRLIMTLTGGETDTSKEVEYTNWNKVSQFAEQFRNW

SEQ ID NO: 11 - protein, 175 aa, The amino acid sequence of PPO11(unclassified Vibrio)
MQKALFLYSSREGQTKKILNYIKEELSEFDCELADLHQIEDIDLALYDRVLIGASIRYGHLNKKLYQFIEKHAEQLALAKAAFFCVNLTARKEAQGKDTPEGSVYIKTFLSKSAWQPKLIGVFAGALYYPRYHFFDKVMIRFIMSLTGGETDTSKEVEYTNWQKVSLFSDNFKKM

SEQ ID NO: 12 - protein, 176 aa, The amino acid sequence of PPO12(Vibrio hepatarius)
MKKALFLYSSREGQTKKILNYIEGELSNFECELVDLHTLDAIDFSVYDRVLIGASIRYGHLNKKLYQFIENNRQQLENHTKVAFFCVNLTARKEDQGKDTPEGSVYIQKFLKKSPWQPKLIGVFAGALYYPRYGFFDKMMIKLIMTLTDGETDTTKEVEYTNWKKVSLFAKKFAEL

SEQ ID NO: 13 - protein, 175 aa, The amino acid sequence of PPO13(Vibrio owensii)
MAKALFLYSSREGQTKKILHYIDEKLTGFECELVDLHNVETIDFSQYDRVLIGASIRYGHLNKKLYQFIDRNLNQLEQSKVAFFCVNLTARKEDQGKDTPEGSAYIRKFLIKSPWKPTLIGVFAGALYYPRYGWFDKTMIKFIMSMTGGETDTTKEVEYTNWEKVALFADKFKEL

SEQ ID NO: 14 - protein, 177 aa, The amino acid sequence of PPO14(Vibrio xiamenensis)
MSNKALLLYSTREGQTKKILQYIDKELHDYQCDYVDLHTMPIEIDFSGYDKVLVGASIRYGHLNKKLYRFIERYKAELKDNNAAFFCVNLTARKEQQGKDTPEGSAYIQTFLKKSPWQPALIGVFAGALRYPKYRWFDKMMIRLIMTMTGGETDTSKEVEYTNWKKVSLFVENWQKQ

SEQ ID NO: 15 - DNA, 537 bp, The nucleotide sequence of PPO1(Ewingella americana)
gagcgtttttttgtacgataacttgccaaaatcctcggcaaacttcttaacttgctcccaatcggtgtattccacttctttactggtatccgtttcgccaccggtcatgcgcataataagttgaatcatgactttatctacccaccgatagcgcggataacgcagcgcgccagcgaatacaccgcacatggcaggtttccatggtgtccccagtaggaacttgcgtacataggagttggtctgaggcgtgcgcttctcaggcttacgcgcagtaaggttcaccgcaaagaacgccgacggcatgctattaagctgttggatattctgttttacaaatttatccagtacggcattgaagtggccgtagcggattgacgcgcccaccagcaccttatcgtagcgagaaagcgtcacatgctgcgcgtgcagcaggtcaatcacatcgcactcatacttctctttcatgcaatttgctatataagaagcaatggcatgtgtttgtccatcacgcgttgaatagagcaccaatgctttcat

SEQ ID NO: 16 - DNA, 522 bp, The nucleotide sequence of PPO2(Vibrio sp. HDW18)
gtgagagcgttattactgtattcaagccaagaagggcaaacgcgtaaaattatccaacgtatcgccgcacagatgccagaatatacttgtgaggtgcaagacttacatcaaagcatcgatattgactgggcggaatacgacaaagtactgattggggcgtcaattcgctatggtcgacttaatcccgccttgtaccgttttattgagcatcacctagtgggattgaccagccgcaaagccgccttcttttgtgtcaatttaaccgctagaaaagaacagcaaggaaaagatactccacagggcagtgcctatatccaaacttttctgaaaaagtcggcttggcagccagagcgaatcgcagtatttgctggcgcgctttattatccacgttaccgctggttcgataaaatgatgatccgcctgatcatgaccttaactggcggcgagaccgatacgagtcaagaagtcgagtataccaactgggataaagtcgttaaatttgctgaacaattccgcaattgg

SEQ ID NO: 17 - DNA, 528 bp, The nucleotide sequence of PPO3(Proteus hauseri)
atgagcgcgctattgctttattgtagtactgatggtcaaacaaaaaaaataatgactcaaattgcgaatgaattaaggcagcatggctatgaatgtgatgtgagagatttaacttctgttcagcagaacttaaatctatctgcttataataaggtattggtcggtgcttctattcgttatggttactttaataaagccttggataaatttataactcgacatctttctcaactcaataatatgccttcagcattctttggcgttaatcttacagcacgaaaagaagaaaagagtacgccagagactaattcttatatatgcaagtttttagataagacaccttggaagccaacattaacaggtgtatttgctggtgcgcttttttaccctcgctataaatggattgatagagtgatgatccaacttattatgaaaatgacaaagggtgaaacagacccaacaaaagaaattgaatatacggattggaataaagttagtgaatttgctactaattttgccaaaataggc

SEQ ID NO: 18 - DNA, 513 bp, The nucleotide sequence of PPO4(Rodentibacter genomosp. 2)
atgaaaacattaattctttattcaagccatgatgggcaaacaaaaaaaatctcggaatttttaaccgcacttttaaatggtgaagtgctggtcgatgctttacgagaagattatgatattgaaacctttgatcaggttattattggcgcttccatacgttatggtcattttagtaaaaccctcgatcgttttgttgttcgtaaccgtgtgcatttggagcaaaaaagagcggtattttttagcgttaatttaactgctcgtaaagagggcaaggataaccccgaaactaatgtatatgtacgcaaatttttacaacgcacaaaatggcagcctaaattggctgcagtgtttgccggagcactattatatccacgctataaatggtttgatcgtgtgatgatacgattcattatgaaaatcactggtggtgagacagatataacaaaagagatcgaatatacggattgggaaaaagtaagggaatttgcccaacggattaacaggttggagaaa

SEQ ID NO: 19 - DNA, 528 bp, The nucleotide sequence of PPO5(Mannheimia pernigra)
aattaactgatcgcttaattttttgccaaactcttccacctgttgccaattcgtatattcatactctttactgacgtctgtttcgcctttagttactttcataataaagcgaatcatcatacggtcaatgaaacgatagcgtgggtagaacaacgccccagcaatcacttcaacatagtttggttgccatttcactttagccaaaaagttacgtatataagtattagtggtaggtgtgttacgatttgctttgcgagcggtcagatttacgccataaaatgccgttttcttttcatttaacatagcataatgctgttcgataaattgataaaccaacggactaaaatgtccataacgaatggaggcaccaatcacaacttgatcaacatttgccattttttgggcaaaatcgaccgcttgatccttaagggagatcagctccacttcgtgtgtgatcacatccgctagtcgctcagcaatctttttcgtttgaccatcggtcgtaaaatagagaattaaggttttcat

SEQ ID NO: 20 - DNA, 693 bp, The nucleotide sequence of PPO6(Leptomonas pyrrhocoris)
atgtcttcaccgaacggaaaatacctgatgttgtactcgacaacagacggccacaccaagacgatcatggacacgatggcgaagcacattatggaagaggcgaaggtgcaatgcgatgtggttgatatgagggacggggacaagtacgaactcgccgcgtacgaaaaggtcatgctcggagcttcgatccggtacggattcttcagcaggacgctgcacacctacaccacacatcacgttgacgagctgaactcgatgccctccgcgttcttcggtgtcaaccttaccgcgaggaagacaagcaaaaacacagcgatgacaaatgcgtacacgcgcaaatttctggaccaatcgatgtgggtgccacaattatcgggggtctttgctggcgctctatggtatccgcggtataacttctttgatcgagtgatgattcaatttatcatgaaagtaaccggcggtgagacaaacacaacaaaagaaattgtctacacggattgggatgcggttcataaatttgctaccgacttcgtacagctaccggcgacggctattcctcgctccaagcccgcgacctcagtgccgccagcgagtgttgcaaactacgataatggtgctcgtgtggcgcttgtcgtcgttggcatttcagcagccattatcttcggtcgccgcctcattctcgcgaaacggttt

SEQ ID NO: 21 - DNA, 522 bp, The nucleotide sequence of PPO7(Aeromonas aquatica)
atggacaagattttggtgctttattcttcccaggacgggcaaacacggaaaattgtggatgccatgctggaggaaatatcaggatgcgacgtggtgatacaggatctgcataccctgcccaagtgcaatctcagcaagtatgccaaggtattgatcggtgcctccattcgctatggcaacttccaccccagcctgctcagcttcatcaatgctcaccatgaacagctggaagtggccaatgccgcattcttctgcgtcaacctgaccgcccgcaagccagagaagcagacgccgcaaaccaatgcctatatgaagaagttcctgcgcctctctccctggaagccgaaaaccctgggggtcttcgccggtgcgctgcaatactcccgctataactggtggcagacccgcatcattcagctgatcatgaagatgaccggcggcagcacggacaccagccaggacctcgagtttaccgattgggtaaaggtacgcagttttgcgcgagaattctggtcaaaaaga

SEQ ID NO: 22 - DNA, 573 bp, The nucleotide sequence of PPO8(Psychromonas sp. SA13A)
acgtgctgcaaagtcctgagcaaaagaatcaactttttcccaatcggttaattctatgtcctgtgttttatcggtactgccgcccgtcattttcataatcaactgaattaacagggtttgccaccaattataacgtgaatacaatagagctccggcaaacacccctttgaactgtggttgccattgtgaaagctgatcaaattttttcatataggcattattttctggcactgctttttctggcttacgtgcagttaaacaaaccacaaaaaaagcattacatactgcatctaattgcgttttatgctgattaacaaacttaattatattgggacgaaagttaccataacgaatagatgcaccgattaagactttttggtacaaagaaaaatcaatggtcggattatcatcaacattcaatacaatcacttcgccagtaagcgtttgcttaatacgattaattatttttaatgtttgtccatcgacagaggaataaagtactaaagttttgcttactacactactttcagtttgcttggtttcagcttgcttagcttgagtttcattagacat

SEQ ID NO: 23 - DNA, 522 bp, The nucleotide sequence of PPO9(Photobacterium aquae)
atagtgcttaaaccgggctgcaaaggcctctactttctgccaatctgtatattcgacttctttactagtatctgtttccccgccagtgatacgcataatgaattgaatcatgacacgatcaaaccatccataccgcggatagcgtaatgccccagcaaatacttcctgcaactttggacaccatggagacttcttcaagaacgttttcatatacacgcttgtctccggcgtattcttaccttccttacgtgccgtaagattcacgcagaaaaaacccaccttattctggtcaagctcatctcggtacctctcgataaactgatagagctttttatttagatggccgtaacgaatagaggctccgaccaatacccgatcataatccgcaaaatccaccgtaggtaatgtgttcaaatcaaccaattcacactggtagtcaccacctagcgtcgtttcgatatgacgtaatattttgacagtctggccatcactgcttgaatgcagcaacaaaactttttccat

SEQ ID NO: 24 - DNA, 522 bp, The nucleotide sequence of PPO10(Vibrio mimicus)
ccaattgcggaattgttcggcaaattgagagactttattccagttagtgtactccacttctttactggtatcggtctctccaccagttagcgtcatgattagacgtatcatcattttatcgaaccaacggtagcgcgggtaatacagcgccccagcaaatacggcgatacgctctggctgccaaggcgactttttcaggaaggtttgaatgtagacactcccttccggcgtatcttttccttgttcttcttttcttgcggtaaggttaacgcaaaagaaggcggctttattactgcgtagatcgggaagataacgctggatgaactggtagagtttgtcgttgaggcggccataacgaatcgatgcaccaatcaagattttgtcgtaatcagctagcgctatgtcacttacctgatgcagatcttggatatcacaatcgtattccggcatctgctgcgcgatgcgttcgataattttccgcgtctgcccttcttggcttgaatacaaaaatagcgctttcac

SEQ ID NO: 25 - DNA, 525 bp, The nucleotide sequence of PPO11(unclassified Vibrio)
catttttttaaagttatcactaaaaagagatactttttgccagtttgtgtactcaacttcttttgaggtgtcagtttcaccgccagtcaatgacatgatgaaacgaatcatcaccttatcgaaaaagtgataacgtggatagtaaagagcaccagcgaaaactccgattagcttgggttgccatgctgatttactgagaaaggttttaatatagacacttccttctggagtatctttaccctgcgcttcttttcttgcagttaagttgacacaaaagaacgccgctttagcgagtgctaattgctcggcatgtttttctataaattgataaagctttttatttaaatgtccgtagcgaatagaagcaccaattaagactcgatcgtaaagagctaaatcaatatcctcaatttgatgtaaatcggcaagttcgcaatcaaactcagaaagttcctcttttatatagttaagaattttcttggtttgaccttcacgggaagaatagagaaaaagagctttttgcac

SEQ ID NO: 26 - DNA, 528 bp, The nucleotide sequence of PPO12(Vibrio hepatarius)
gtgaaaaaagctttatttctgtattcttcacgcgaaggtcaaaccaaaaagattcttaactatatagagggtgagcttagcaacttcgaatgtgagctggttgacctacatacattagacgcaatagatttcagcgtttatgacagagtgctgattggggcttcgatccgatacggacatttaaataagaaactctatcagtttatcgagaacaatcgacaacaactggaaaatcacactaaggtggcatttttctgcgttaacttgaccgcgcgtaaggaagaccaaggtaaagatacccctgaaggcagcgtttatattcagaagtttttaaagaaatcgccttggcaacctaagttaatcggggtattcgccggggctttatattacccgcgctatggtttcttcgacaaaatgatgattaaactgattatgacgctgaccgatggtgaaacggatactactaaagaagtcgagtacaccaattggaaaaaggtctctcttttcgcgaaaaaattcgctgagttg

SEQ ID NO: 27 - DNA, 528 bp, The nucleotide sequence of PPO13(Vibrio owensii)
gtggcaaaagcattatttctatattcctcccgtgaagggcagactaaaaaaattctccactatatagatgagaagctaacaggcttcgaatgtgagctggtggatttacataatgttgagacgattgattttagccaatacgacagggtattgattggagcgtctattcgttatggtcatcttaataagaagctgtaccagtttattgatcgaaacctcaatcagcttgaacaaagtaaagtggcatttttctgcgtaaacctaaccgctcgtaaagaagaccaaggaaaggatacgccagagggcagcgcttacattcgtaagttcctaattaagtcaccttggaaaccaaccttaatcggtgtttttgctggtgctctttattacccacgttacggatggttcgacaaaacgatgattaagttcattatgtcgatgacgggtggcgaaaccgatacgaccaaagaagtggaatacaccaattgggaaaaagtggctcttttcgcagataaattcaaagaactgtag

SEQ ID NO: 28 - DNA, 531 bp, The nucleotide sequence of PPO14(Vibrio xiamenensis)
ttgagtaacaaagcgctattgctttattcaacgcgagaagggcaaaccaagaaaattctccaatacatagataaagagctgcacgactatcagtgcgattacgttgacttacataccatgccaatagagatagatttctctggttatgacaaagtgctggtgggggcttctattcgttatgggcatctcaacaaaaaactgtatcggtttattgagcgttataaagccgaattgaaagacaacaacgcggcgttcttttgcgttaatttaacggcgcgcaaagaacagcaaggaaaagataccccagagggcagcgcttatattcaaacctttcttaagaagtccccatggcaaccagcattgattggtgtgtttgctggggcattgcgctatccgaagtaccgttggtttgacaaaatgatgattcgtttgatcatgaccatgacaggtggtgaaacggataccagtaaagaagtcgaatatacaaactggaaaaaagtctctctttttgtcgaaaattggcaaaaacag

SEQ ID NO: 29 - DNA, 540 bp, The nucleotide sequence of PPO1A(Artificial Sequence)
atgaaggctttggtactctacagcacaagagacggtcagacacacgcgatcgcgtcgtacattgctaattgcatgaaagagaagtatgagtgtgacgttattgatcttcttcatgctcagcatgttacattatcacggtatgataaggttcttgtaggagcttctatacgatatggacatttcaatgctgtgttggacaaatttgtgaagcaaaacatccaacaactaaactcaatgccttctgctttctttgctgttaatttgactgccaggaaacctgagaaacgtactcctcagaccaattcttatgttaggaagtttcttctggggacaccatggaaaccagcaatgtgtggcgtgtttgcaggagcattgaggtatccacgttacagatgggttgataaagtgatgattcagctcataatgagaatgactggtggtgaaacagatacaagcaaagaagttgagtatactgattgggaacaagtcaaaaagttcgcagaagattttggaaagctaagttacaagaaaaccctctga

SEQ ID NO: 30 - DNA, 525 bp, The nucleotide sequence of PPO2A(Artificial Sequence)
atgagagccttgcttctctacagcagtcaagaagggcagacaagaaaaatcattcagagaatagcagctcaaatgcctgagtacacttgtgaagttcaagatttgcatcaatcaatagatattgattgggccgagtatgacaaagttttaattggtgcatccatccggtatggacgtttgaaccctgcactttacaggttcattgagcatcacctcgttggtttgacctcaaggaaggctgctttcttctgcgtaaatcttaccgcaaggaaagaacaacaagggaaagacactccacagggctctgcatatattcaaacatttttgaagaagagtgcttggcaacccgaaaggattgctgtttttgctggtgccctttattatccaagatacagatggtttgataagatgatgatccgactcatcatgacgttaactggaggagaaactgatacatctcaggaggtggaatatacaaactgggataaagtcgtgaagtttgcagagcagtttcggaattggtga

SEQ ID NO: 31 - DNA, 531 bp, The nucleotide sequence of PPO3A(Artificial Sequence)
atgagtgccctgttgttgtattgttcaactgatggtcaaaccaagaagataatgacacagatagctaatgaactgagacaacatggttatgaatgtgatgtgcgggatcttacttctgttcaacaaaatctcaatctttcagcttacaacaaagttttggtaggagcttccataagatatggatacttcaataaagcacttgacaagttcatcacgaggcacctctctcagttaaacaacatgccttctgctttctttggtgtcaatttgactgcaagaaaagaagagaagagcactcccgaaacaaacagttacatctgcaagtttctagacaaaacaccatggaaaccaaccttaactggagtcttcgccggggcgcttttttatcctcgttacaaatggattgatcgagtgatgattcagcttatcatgaagatgactaaaggagaaaccgatccgacaaaagagattgagtatacagattggaacaaggtttcggagtttgctacgaattttgcaaagattggctga

SEQ ID NO: 32 - DNA, 516 bp, The nucleotide sequence of PPO4A(Artificial Sequence)
atgaaaaccctgattctttacagcagtcatgatggacagaccaagaaaatctcagagttccttacggcgttgttgaatggcgaagttctagttgatgctctacgtgaagattatgatattgaaacatttgaccaagttataatcggagcttccataaggtatggtcacttttctaagactttagacagatttgtggtgagaaacagggtacatctggaacaaaaacgagcagtattcttctctgttaacttaactgcccgaaaagaaggtaaagacaatcctgaaactaatgtctatgtcagaaagtttctccagagaacaaaatggcaaccaaaacttgctgccgtcttcgcaggtgcactcttgtacccgagatataagtggtttgatcgtgtgatgattcggtttatcatgaagattactgggggagagacggatataacaaaggagattgagtacacagattgggaaaaggttagggagttcgctcagagaatcaaccgccttgagaaatga

SEQ ID NO: 33 - DNA, 531 bp, The nucleotide sequence of PPO5A(Artificial Sequence)
atgaagactcttatcctctacttcacaacagacggccaaacgaaaaagattgccgagagactggctgatgtgattactcatgaagtggagctaatctccttgaaagatcaagctgttgattttgctcagaagatggctaatgttgaccaagtagtcattggagcgagtataaggtatggtcacttcagccctcttgtttatcagtttattgaacaacattatgcaatgttgaatgagaagaaaaccgctttttatggagtgaatctcacagcaaggaaagcaaatcgaaacaccccaaccacaaatacttacatccggaacttcttagcaaaggtgaaatggcaacctaactatgttgaggtcatagctggtgccttgttttacccgcgttacagattcattgatagaatgatgattcgcttcatcatgaaagtaacgaaaggagaaactgatgtttcaaaagaatatgaatacacaaactggcagcaagttgaagagtttgggaagaagctttctgatcagttaatatga

SEQ ID NO: 34 - DNA, 696 bp, The nucleotide sequence of PPO6A(Artificial Sequence)
atgtcttctcctaatgggaagtatttgatgctttacagtaccaccgacggtcacacaaaaaccattatggatacaatggctaaacatataatggaagaagcaaaagtacaatgtgatgttgtggacatgagagatggagacaaatacgagttagctgcttatgagaaggtgatgctaggagcttctattagatatggattcttcagccgcactcttcatacatataccactcatcatgttgatgaacttaactcaatgccttccgctttctttggagtcaatctcactgctcgtaaaacttcaaagaacactgcaatgactaatgcatacacaagaaagtttctggatcaatccatgtgggttcctcaattatctggcgtttttgctggtgctttgtggtatcctaggtacaatttctttgacagggttatgattcagttcatcatgaaggtaactggtggtgaaacaaacacaacgaaagagatagtttacactgattgggatgctgttcacaaatttgcaacagattttgtgcagctaccagccacggcgataccccggagcaagccggcgacgtcggtcccaccagctagtgtggccaactatgataatggggcacgagtagcgcttgtggttgtgggaatctcagcagccatcatctttggccgtcgattgattctcgcaaagagattctga

SEQ ID NO: 35 - DNA, 525 bp, The nucleotide sequence of PPO7A(Artificial Sequence)
atggataagatattagtcctgtacagtagtcaagatgggcagacgaggaagattgttgatgcaatgcttgaagaaatctctggttgtgatgttgtgattcaagacttgcacacactaccgaaatgcaacctatccaaatatgcgaaagtgttgattggtgcttccataaggtatggaaacttccatccttctcttctcagcttcatcaatgctcatcatgaacaacttgaggttgctaatgcggccttcttctgtgtaaatctcactgcccgaaaacctgagaagcaaactccccagacaaacgcttacatgaagaagtttttacgcttatcaccatggaaaccaaagacccttggagtgtttgcaggagctttgcaatattcaagatacaattggtggcaaacccgtatcattcagctgataatgaaaatgactggtggctcaacagacacatctcaggatttggagtttactgattgggttaaagtccggtcgtttgcaagagaattttggagcaagagatga

SEQ ID NO: 36 - DNA, 576 bp, The nucleotide sequence of PPO8A(Artificial Sequence)
atgtcaaatgagacacaagccaaacaagctgaaacgaaacagactgagtcttctgtcgtaagcaaaacgctggtgttgtactcgtccgtcgatggtcaaaccttaaagatcattaatcgtattaagcagaccctgacaggagaagttattgttttgaatgttgatgataatccaactatcgattttagcctttatcagaaggtcttgattggagcatcaatccggtatgggaactttagaccgaacatcataaagtttgttaatcagcataaaacacaacttgacgcggtgtgcaacgctttcttcgtggtttgtctcacagcaagaaaaccagagaaagctgttcctgaaaacaatgcatacatgaagaaatttgatcagctaagtcaatggcaacctcagttcaagggagtattcgcgggtgctttattgtattcacgatacaactggtggcagacacttctcatacaactaataatgaagatgactggtggcagtactgacaaaactcaagatattgagcttaccgattgggaaaaggtggattctttcgcacaagactttgctgccaggtga

SEQ ID NO: 37 - DNA, 525 bp, The nucleotide sequence of PPO9A(Artificial Sequence)
atggagaaagttcttctactgcattcttcctctgatggtcagacagtgaagattctcagacatattgaaacaacattaggtggtgattaccaatgtgagcttgtggatttgaatactctgccgactgttgattttgctgattatgaccgtgtcttagtaggcgcgagtatacgctatgggcacctcaacaagaaactctaccagtttatagagagatacagagatgaattggaccaaaacaaagtaggtttcttctgcgtgaatcttactgcaaggaaagaaggaaagaatacgcctgagactagcgtttacatgaagacctttttgaagaagtcgccatggtgtccaaaattgcaagaagttttcgctggagctcttcgttatcctcggtatggatggtttgatagggtcatgattcagttcatcatgagaatcacggggggagaaaccgacacatcaaaagaggttgagtatactgattggcaaaaggttgaagcttttgcagcccgattcaaacattactga

SEQ ID NO: 38 - DNA, 525 bp, The nucleotide sequence of PPO10A(Artificial Sequence)
atgaaagctctctttctgtactcgtctcaagaaggacagacaaggaagattatagagagaatcgcccagcaaatgccggagtatgattgtgatattcaagatcttcatcaagtaagcgacattgcattagctgattatgacaagatcctaataggggccagtatccgatatggaagattgaatgataaactatatcaatttattcagagatatcttcccgatctccgctccaacaaagcagctttcttctgcgtcaatcttacggcgagaaaggaagaacaaggaaaagacaccccagaaggttctgtttacatccagactttcttgaagaaatcaccatggcaacctgagaggattgcagtgtttgctggtgctctttactatcctcgttacagatggtttgataagatgatgattcggttaataatgactttgaccggcggtgaaactgatacatcaaaagaagttgagtacacaaattggaacaaggtttctcagtttgcggagcagttccgtaactggtga

SEQ ID NO: 39 - DNA, 528 bp, The nucleotide sequence of PPO11A(Artificial Sequence)
atgcaaaaagctcttttcctctacagttcaagagaaggacaaacaaagaaaatactcaactacatcaaggaagaactatcagagtttgattgtgagcttgctgatcttcatcagattgaagatattgatttagccttgtatgatcgagtattaataggcgcaagcatccggtatggtcacttgaacaaaaagctttatcagtttattgagaagcatgctgagcaacttgcgctggcaaaagcagctttcttctgcgtgaatctcactgcaaggaaagaggctcaaggaaaagatactccggaaggttctgtttacataaagacgtttctgtccaagtctgcttggcaaccaaagttgattggagtttttgctggtgccctatactatcctcgttaccatttctttgacaaagtgatgattagattcatcatgtctttaaccgggggagaaactgacacatcaaaagaagttgagtatacaaattggcagaaagtctcgttgtttagtgacaatttcaagaagatgtga

SEQ ID NO: 40 - DNA, 531 bp, The nucleotide sequence of PPO12A(Artificial Sequence)
atgaagaaagctcttttcctgtacagctcgagagaaggccagacaaaaaagattctcaactacatagaaggagagttatcaaattttgaatgtgaattggttgaccttcacacgcttgatgctattgatttctccgtctatgatcgggtgctcattggtgcttctatacgatatggtcatttgaacaagaagctttatcagtttatagagaacaacagacaacaactagagaatcataccaaagttgccttcttctgcgtcaatcttactgcaaggaaagaagatcaaggaaaagacactcctgaggggagtgtttacatccagaaatttctcaagaaatcaccatggcaaccgaagttgattggagttttcgcgggggcattatactaccctcgttatggattctttgataagatgatgatcaaactcatcatgactttaactgatggtgaaaccgacacaacaaaggaagtggagtatacaaattggaaaaaagtatctttgtttgcaaagaagtttgctgagctgtga

SEQ ID NO: 41 - DNA, 528 bp, The nucleotide sequence of PPO13A(Artificial Sequence)
atggctaaagctcttttcctgtactcatctagagaaggacaaacaaagaagattcttcattacatagacgagaagttaactgggtttgagtgtgaactcgttgatttgcacaatgtcgaaactattgatttttctcagtatgatagagtcttaattggagcgtccatacgatatggtcatctcaacaagaaattatatcagtttatcgaccgtaacctgaaccagctagagcaaagcaaggtagctttcttctgcgtgaatctcaccgcacggaaagaggatcaaggaaaagatactcctgaaggctcagcttacataaggaagtttcttatcaaatcgccttggaaaccgacattgattggtgttttcgcaggtgcactttactatccaagatatgggtggtttgataaaacaatgatcaaattcatcatgagtatgactggtggagaaaccgacacgaccaaggaagttgagtacacaaattgggaaaaagtggccttgtttgctgataagttcaaggagctatga

SEQ ID NO: 42 - DNA, 534 bp, The nucleotide sequence of PPO14A(Artificial Sequence)
atgtctaacaaggccttgctgctctatagtacaagagaaggtcaaactaaaaagattcttcagtacatagacaaagagcttcatgattaccaatgtgattatgtcgatcttcacacaatgcctatagagattgatttctctggttatgataaagttttggtaggggcgtccatccggtatggacatttaaacaaaaaactttacagattcatcgagaggtacaaagcagagttgaaggataataatgctgctttcttctgcgtcaatctaaccgcaaggaaagaacaacaaggaaaagatactcctgaaggatcagcttatattcagacttttctcaagaagtctccatggcagccagcattgataggtgtttttgctggagctttacgttacccgaagtatagatggtttgacaagatgatgattcgactaatcatgactatgacgggcggtgaaaccgacacatcaaaggaagtggagtatacaaattggaagaaagtgagcctctttgttgaaaactggcaaaagcagtga

SEQ ID NO: 43 - protein, 181 aa, The amino acid sequence of PPO-EC(Escherichia coli)
MKTLILFSTRDGQTREIASYLASELKELGIQADVANVHRIEEPQWENYDRVVIGASIRYGHYHSAFQEFVKKHATRLNSMPSAFYSVNLVARKPEKRTPQTNSYARKFLMNSQWRPDRCAVIAGALRYPRYRWYDRFMIKLIMKMSGGETDTRKEVVYTDWEQVANFAREIAHLTDKPTLK

SEQ ID NO: 44 - DNA, 546 bp, The nucleotide sequence of PPO-EC(Escherichia coli)
gtgaaaacattaattcttttctcaacaagggacggacaaacgcgcgagattgcctcctacctggcttcggaactgaaagaactggggatccaggcggatgtcgccaatgtgcaccgcattgaagaaccacagtgggaaaactatgaccgtgtggtcattggtgcttctattcgctatggtcactaccattcagcgttccaggaatttgtcaaaaaacatgcgacgcggctgaattcgatgccgagcgccttttactccgtgaatctggtggcgcgcaaaccggagaagcgtactccacagaccaacagctacgcgcgcaagtttctgatgaactcgcaatggcgtcccgatcgctgcgcggtcattgccggggcgctgcgttacccacgttatcgctggtacgaccgttttatgatcaagctgattatgaagatgtcaggcggtgaaacggatacgcgcaaagaagttgtctataccgattgggagcaggtggcgaatttcgcccgagaaatcgcccatttaaccgacaaaccgacgctgaaataa

SEQ ID NO: 45 - DNA, 546 bp, The nucleotide sequence of PPO-ECA(Artificial Sequence)
atgaaaacacttatcttgttctcaactagagatggacagacaagagagattgcttcttacttggcttcagaacttaaggagttgggtattcaagctgatgttgctaatgttcatagaattgaagagcctcagtgggaaaactatgatagagttgttattggagcttctattagatatggtcattaccattcagcttttcaagagttcgttaagaaacatgctactagacttaactctatgccatcagctttttactctgttaacttggttgctagaaagcctgagaaaagaactccacaaacaaactcttacgctagaaagttccttatgaactcacagtggagacctgatagatgcgctgttattgctggtgctcttagatatccaagatacagatggtacgatagattcatgatcaagttgattatgaaaatgtctggaggtgaaactgatacaagaaaggaggttgtttacacagattgggaacaggttgctaatttcgctagagagattgctcatcttactgataagccaacattgaaatga

SEQ ID NO: 46 - protein, 537 aa, The amino acid sequence of PPO-AT(Arabidopsis thaliana)
MELSLLRPTTQSLLPSFSKPNLRLNVYKPLRLRCSVAGGPTVGSSKIEGGGGTTITTDCVIVGGGISGLCIAQALATKHPDAAPNLIVTEAKDRVGGNIITREENGFLWEEGPNSFQPSDPMLTMVVDSGLKDDLVLGDPTAPRFVLWNGKLRPVPSKLTDLPFFDLMSIGGKIRAGFGALGIRPSPPGREESVEEFVRRNLGDEVFERLIEPFCSGVYAGDPSKLSMKAAFGKVWKLEQNGGSIIGGTFKAIQERKNAPKAERDPRLPKPQGQTVGSFRKGLRMLPEAISARLGSKVKLSWKLSGITKLESGGYNLTYETPDGLVSVQSKSVVMTVPSHVASGLLRPLSESAANALSKLYYPPVAAVSISYPKEAIRTECLIDGELKGFGQLHPRTQGVETLGTIYSSSLFPNRAPPGRILLLNYIGGSTNTGILSKSEGELVEAVDRDLRKMLIKPNSTDPLKLGVRVWPQAIPQFLVGHFDILDTAKSSLTSSGYEGLFLGGNYVAGVALGRCVEGAYETAIEVNNFMSRYAYK

SEQ ID NO: 47 - DNA, 1614 bp, The nucleotide sequence of PPO-AT(Arabidopsis thaliana)
atggagttatctcttctccgtccgacgactcaatcgcttcttccgtcgttttcgaagcccaatctccgattaaatgtttataagcctcttagactccgttgttcagtggccggtggaccaaccgtcggatcttcaaaaatcgaaggcggaggaggcaccaccatcacgacggattgtgtgattgtcggcggaggtattagtggtctttgcatcgctcaggcgcttgctactaagcatcctgatgctgctccgaatttaattgtgaccgaggctaaggatcgtgttggaggcaacattatcactcgtgaagagaatggttttctctgggaagaaggtcccaatagttttcaaccgtctgatcctatgctcactatggtggtagatagtggtttgaaggatgatttggtgttgggagatcctactgcgccaaggtttgtgttgtggaatgggaaattgaggccggttccatcgaagctaacagacttaccgttctttgatttgatgagtattggtgggaagattagagctggttttggtgcacttggcattcgaccgtcacctccaggtcgtgaagaatctgtggaggagtttgtacggcgtaacctcggtgatgaggtttttgagcgcctgattgaaccgttttgttcaggtgtttatgctggtgatccttcaaaactgagcatgaaagcagcgtttgggaaggtttggaaactagagcaaaatggtggaagcataataggtggtacttttaaggcaattcaggagaggaaaaacgctcccaaggcagaacgagacccgcgcctgccaaaaccacagggccaaacagttggttctttcaggaagggacttcgaatgttgccagaagcaatatctgcaagattaggtagcaaagttaagttgtcttggaagctctcaggtatcactaagctggagagcggaggatacaacttaacatatgagactccagatggtttagtttccgtgcagagcaaaagtgttgtaatgacggtgccatctcatgttgcaagtggtctcttgcgccctctttctgaatctgctgcaaatgcactctcaaaactatattacccaccagttgcagcagtatctatctcgtacccgaaagaagcaatccgaacagaatgtttgatagatggtgaactaaagggttttgggcaattgcatccacgcacgcaaggagttgaaacattaggaactatctacagctcctcactctttccaaatcgcgcaccgcccggaagaattttgctgttgaactacattggcgggtctacaaacaccggaattctgtccaagtctgaaggtgagttagtggaagcagttgacagagatttgaggaaaatgctaattaagcctaattcgaccgatccacttaaattaggagttagggtatggcctcaagccattcctcagtttctagttggtcactttgatatccttgacacggctaaatcatctctaacgtcttcgggctacgaagggctatttttgggtggcaattacgtcgctggtgtagccttaggccggtgtgtagaaggcgcatatgaaaccgcgattgaggtcaacaacttcatgtcacggtacgcttacaagtaa

SEQ ID NO: 48 - DNA, 1614 bp, The nucleotide sequence of PPO-ATA(Artificial Sequence)
atggagttgtctcttttaagaccaacaacacaatctttgcttccttcgttctctaaacccaatctcagattgaatgtctacaaaccactacgattgcgatgctctgtggctggtggtcctactgttggaagttcaaagatagaaggaggcggtggtacaaccatcactacagattgtgtgattgtaggtggtggcatttcgggtctttgcattgctcaagctctcgctacaaaacatcctgacgctgcgcccaacttaatagtgacggaagcaaaagacagagttggtgggaatattatcacaagagaagagaatgggtttttatgggaagaaggaccgaacagctttcaaccgtcagatccaatgcttacaatggtggttgattctggactgaaagatgatctcgtacttggtgatccgacggccccaaggtttgttttgtggaatggaaaattgcgacctgttccaagcaaattaacagatttacctttcttcgatctcatgagtataggtgggaagatcagggccggttttggtgcactgggaatccgtccttctcctcctggaagagaggagagcgtagaagagtttgtgcgtaggaacctgggagatgaagtttttgagaggttgattgagccattttgctcaggcgtttatgcaggtgacccgagcaagctgtctatgaaggctgctttcggcaaagtttggaagctcgagcagaatggtggatctattattggaggaactttcaaggccattcaagaaagaaagaatgctcctaaagcagagagggaccctagacttcccaagcctcaaggacaaaccgtcggctctttcaggaaaggattaagaatgttgccagaggctatcagtgcgcgccttggaagcaaggttaaactttcatggaaactatctgggataaccaaacttgaatcaggaggttacaatttaacttatgaaactccggatggacttgtttctgtacagagtaagtcagttgtgatgacggttccttcacatgtcgcttctggtctgttgcgtccattatccgaatctgccgctaatgcattatccaaactctactatcctcccgtggcagcagtcagtatctcttatccaaaagaagctattagaacagaatgtcttattgatggtgagcttaagggatttggacagcttcaccctcgaactcagggtgtggaaacactggggactatttatagttcctccttgtttcctaaccgtgcaccacctgggagaattcttcttctaaactacattggagggtcaacaaacaccggtatcctatcgaagagtgagggagaattagttgaagctgtcgacagagacctaaggaagatgctgataaagccaaattcaaccgaccccctcaagctcggagttcgcgtgtggcctcaggcaattccgcaattcctggtaggacattttgatatattggatactgccaaatcttctcttacttcatcgggctacgaaggtttgtttcttggcggaaactatgttgctggagttgccttggggcgctgtgtagagggtgcttatgagactgcaatagaggtgaacaatttcatgtctagatatgcttacaagtga

SEQ ID NO: 49 - DNA, 21 bp, 5'end universal adapter primer 1(Artificial Sequence)
taagaaggagatatacatatg

SEQ ID NO: 50 - DNA, 21 bp, 3'end universal adapter primer 1(Artificial Sequence)
gtggtggtggtggtgctcgag

SEQ ID NO: 51 - DNA, 542 bp, 34S enhancer(Figwort mosaic virus)
aattctcagtccaaagcctcaacaaggtcagggtacagagtctccaaaccattagccaaaagctacaggagatcaatgaagaatcttcaatcaaagtaaactactgttccagcacatgcatcatggtcagtaagtttcagaaaaagacatccaccgaagacttaaagttagtgggcatctttgaaagtaatcttgtcaacatcgagcagctggcttgtggggaccagacaaaaaaggaatggtgcagaattgttaggcgcacctaccaaaagcatctttgcctttattgcaaagataaagcagattcctctagtacaagtggggaacaaaataacgtggaaaagagctgtcctgacagcccactcactaatgcgtatgacgaacgcagtgacgaccacaaaagaattagcttgagctcaggatttagcagcattccagattgggttcaatcaacaaggtacgagccatatcactttattcaaattggtatcgccaaaaccaagaaggaactcccatcctcaaaggtttgtaaggaagaattc

SEQ ID NO: 52 - DNA, 1534 bp, Promoter of Oilseed rape eukaryotic elongation factor gene 1a (Tsf1,Brassica napus)
gattatgacattgctcgtggaatgggacagttatggtatttttttgtaataaattgtttccattgtcatgagattttgaggttaatctatgagacattgaatcacttagcattagggattaagtagtcacaaatcgcattcaagaagctgaagaacacgttatggtctaatggttgtgtctctttattagaaaatgttggtcagtagctatatgcactgtttctgtaaaaccatgttggtgttgtgtttatttcaagacacatgttgagtccgttgattcagagcttttgtcttcgaacacaatctagagagcaaatttgggttcaatttggatatcaatatgggttcgattcagatagaacaataccctttgatgtcgggtttcgatttggttgagattcatttttatcgggtttggttcgattttcgaattcggtttattcgccccctcatagcatctacattctgcagattaatgtacaagttatggaaaaaaaaatgtggttttcgaattcggtttagtagctaaacgttgcttgcagtgtagttatgggaattatgaaacacgaccgaaggtatcaattagaagaacgggtcaacgggtaagtattgagaaattaccggagggtaaaaataaacagtattctttttttttcttaacgaccgaccaaggttaaaaaaagaaaggaggacgagatacaggggcatgactgtaattgtacataagatctgatctttaaaccctaggtttccttcgcatcagcaactataaataattctgagtgccactcttcttcattcctagatctttcgccttatcgctttagctgaggtaagcctttctatacgcatagacgctctcttttctcttctctcgatcttcgttgaaacggtcctcgatacgcataggatcggttagaatcgttaatctatcgtcttagatcttcttgattgttgaattgagcttctaggatgtattgtatcatgtgatggatagttgattggatctctttgagtgaactagctagctttcgatgcgtgtgatttcagtataacaggatccgatgaattatagctcgcttacaattaatctctgcagatttattgtttaatcttggatttgatgctcgttgttgatagaggatcgtttatagaacttattgattctggaattgagcttgtgtgatgtattgtatcatgtgatcgatagctgatggatctatttgagtgaactagcgtacgatcttaagatgagtgtgtattgtgaactgatgattcgagatcagcaaaacaagatctgatgatatcttcgtcttgtatgcatcttgaatttcatgattttttattaattatagctcgcttagctcaaaggatagagcaccacaaaattttattgtggtagaaatcggttcgattccgatagcagcttactgtgatgaatgattttgagatttggtatttgatatatgtctactgtgttgaatgatcgtttatgcattgtttaatcgctgcagatttgcattgacaagtagcc

SEQ ID NO: 53 - DNA, 228 bp, Chloroplast transit peptide(Arabidopsis thaliana)
atggcgcaagttagcagaatctgcaatggtgtgcagaacccatctcttatctccaatctctcgaaatccagtcaacgcaaatctcccttatcggtttctctgaagacgcagcagcatccacgagcttatccgatttcgtcgtcgtggggattgaagaagagtgggatgacgttaattggctctgagcttcgtcctcttaaggtcatgtcttctgtttccacggcgtgc

SEQ ID NO: 54 - DNA, 1368 bp, 5-enolpyruvylshikimate-3-phosphate synthase gene (Artificial Sequence)
atgcttcacggtgcaagcagccgtccagcaactgctcgtaagtcctctggtctttctggaaccgtccgtattccaggtgacaagtctatctcccacaggtccttcatgtttggaggtctcgctagcggtgaaactcgtatcaccggtcttttggaaggtgaagatgttatcaacactggtaaggctatgcaagctatgggtgccagaatccgtaaggaaggtgatacttggatcattgatggtgttggtaacggtggactccttgctcctgaggctcctctcgatttcggtaacgctgcaactggttgccgtttgactatgggtcttgttggtgtttacgatttcgatagcactttcattggtgacgcttctctcactaagcgtccaatgggtcgtgtgttgaacccacttcgcgaaatgggtgtgcaggtgaagtctgaagacggtgatcgtcttccagttaccttgcgtggaccaaagactccaacgccaatcacctacagggtacctatggcttccgctcaagtgaagtccgctgttctgcttgctggtctcaacaccccaggtatcaccactgttatcgagccaatcatgactcgtgaccacactgaaaagatgcttcaaggttttggtgctaaccttaccgttgagactgatgctgacggtgtgcgtaccatccgtcttgaaggtcgtggtaagctcaccggtcaagtgattgatgttccaggtgatccatcctctactgctttcccattggttgctgccttgcttgttccaggttccgacgtcaccatccttaacgttttgatgaacccaacccgtactggtctcatcttgactctgcaggaaatgggtgccgacatcgaagtgatcaacccacgtcttgctggtggagaagacgtggctgacttgcgtgttcgttcttctactttgaagggtgttactgttccagaagaccgtgctccttctatgatcgacgagtatccaattctcgctgttgcagctgcattcgctgaaggtgctaccgttatgaacggtttggaagaactccgtgttaaggaaagcgaccgtctttctgctgtcgcaaacggtctcaagctcaacggtgttgattgcgatgaaggtgagacttctctcgtcgtgcgtggtcgtcctgacggtaagggtctcggtaacgcttctggagcagctgtcgctacccacctcgatcaccgtatcgctatgagcttcctcgttatgggtctcgtttctgaaaaccctgttactgttgatgatgctactatgatcgctactagcttcccagagttcatggatttgatggctggtcttggagctaagatcgaactctccgacactaaggctgcttga

SEQ ID NO: 55 - DNA, 643 bp, Terminator of a pea RbcS gene(Pisum sativum)
agctttcgttcgtatcatcggtttcgacaacgttcgtcaagttcaatgcatcagtttcattgcgcacacaccagaatcctactgagtttgagtattatggcattgggaaaactgtttttcttgtaccatttgttgtgcttgtaatttactgtgttttttattcggttttcgctatcgaactgtgaaatggaaatggatggagaagagttaatgaatgatatggtccttttgttcattctcaaattaatattatttgttttttctcttatttgttgtgtgttgaatttgaaattataagagatatgcaaacattttgttttgagtaaaaatgtgtcaaatcgtggcctctaatgaccgaagttaatatgaggagtaaaacacttgtagttgtaccattatgcttattcactaggcaacaaatatattttcagacctagaaaagctgcaaatgttactgaatacaagtatgtcctcttgtgttttagacatttatgaactttcctttatgtaattttccagaatccttgtcagattctaatcattgctttataattatagttatactcatggatttgtagttgagtatgaaaatattttttaatgcattttatgacttgccaattgattgacaacatgcatcaat

SEQ ID NO: 56 - DNA, 1322 bp, Promoter of Ubiquitin 10 gene(Arabidopsis thaliana)
gtcgacctgcaggtcaacggatcaggatattcttgtttaagatgttgaactctatggaggtttgtatgaactgatgatctaggaccggataagttcccttcttcatagcgaacttattcaaagaatgttttgtgtatcattcttgttacattgttattaatgaaaaaatattattggtcattggactgaacacgagtgttaaatatggaccaggccccaaataagatccattgatatatgaattaaataacaagaataaatcgagtcaccaaaccacttgccttttttaacgagacttgttcaccaacttgatacaaaagtcattatcctatgcaaatcaataatcatacaaaaatatccaataacactaaaaaattaaaagaaatggataatttcacaatatgttatacgataaagaagttacttttccaagaaattcactgattttataagcccacttgcattagataaatggcaaaaaaaaacaaaaaggaaaagaaataaagcacgaagaattctagaaaatacgaaatacgcttcaatgcagtgggacccacggttcaattattgccaattttcagctccaccgtatatttaaaaaataaaacgataatgctaaaaaaatataaatcgtaacgatcgttaaatctcaacggctggatcttatgacgaccgttagaaattgtggttgtcgacgagtcagtaataaacggcgtcaaagtggttgcagccggcacacacgagtcgtgtttatcaactcaaagcacaaatacttttcctcaacctaaaaataaggcaattagccaaaaacaactttgcgtgtaaacaacgctcaatacacgtgtcattttattattagctattgcttcaccgccttagctttctcgtgacctagtcgtcctcgtcttttcttcttcttcttctataaaacaatacccaaagcttcttcttcacaattcagatttcaatttctcaaaatcttaaaaactttctctcaattctctctaccgtgatcaaggtaaatttctgtgttccttattctctcaaaatcttcgattttgttttcgttcgatcccaatttcgtatatgttctttggtttagattctgttaatcttagatcgaagacgattttctgggtttgatcgttagatatcatcttaattctcgattagggtttcataaatatcatccgatttgttcaaataatttgagttttgtcgaataattactcttcgatttgtgatttctatctagatctggtgttagtttctagtttgtgcgatcgaatttgtcgattaatctgagtttttctgattaacag

SEQ ID NO: 57 - DNA, 234 bp, Albino or pale-green chloroplast transit peptide (Arabidopsis thaliana)
atggctacagctactacaactgctactgctgctttttcaggagttgtttctgttggtacagaaactagaagaatctattcattctctcatcttcaaccttcagctgcttttcctgctaagccatcttcattcaaatcacttaagttgaagcagtctgctagacttacaagaagattggatcatagaccatttgttgttagatgtgaggcttcttcatctaacggaagacttact

SEQ ID NO: 58 - DNA, 253 bp, Terminator of nopaline synthetase gene(Agrobacterium tumefaciens)
gatcgttcaaacatttggcaataaagtttcttaagattgaatcctgttgccggtcttgcgatgattatcatataatttctgttgaattacgttaagcatgtaataattaacatgtaatgcatgacgttatttatgagatgggtttttatgattagagtcccgcaattatacatttaatacgcgatagaaaacaaaatatagcgcgcaaactaggataaattatcgcgcgcggtgtcatctatgttactagatc

SEQ ID NO: 59 - DNA, 530 bp, 35S promoter(Cauliflower mosaic virus)
ccatggagtcaaagattcaaatagaggacctaacagaactcgccgtaaagactggcgaacagttcatacagagtctcttacgactcaatgacaagaagaaaatcttcgtcaacatggtggagcacgacacgcttgtctactccaaaaatatcaaagatacagtctcagaagaccaaagggcaattgagacttttcaacaaagggtaatatccggaaacctcctcggattccattgcccagctatctgtcactttattgtgaagatagtggaaaaggaaggtggctcctacaaatgccatcattgcgataaaggaaaggccatcgttgaagatgcctctgccgacagtggtcccaaagatggacccccacccacgaggagcatcgtggaaaaagaagacgttccaaccacgtcttcaaagcaagtggattgatgtgatatctccactgacgtaagggatgacgcacaatcccactatccttcgcaagacccttcctctatataaggaagttcatttcatttggagaggaca

SEQ ID NO: 60 - DNA, 552 bp, Phosphinothricin-N-acetyl-transferase gene (Streptomyces viridochromogenes)
atgtctccggagaggagaccagttgagattaggccagctacagcagctgatatggccgcggtttgtgatatcgttaaccattacattgagacgtctacagtgaactttaggacagagccacaaacaccacaagagtggattgatgatctagagaggttgcaagatagatacccttggttggttgctgaggttgagggtgttgtggctggtattgcttacgctgggccctggaaggctaggaacgcttacgattggacagttgagagtactgtttacgtgtcacataggcatcaaaggttgggcctaggatccacattgtacacacatttgcttaagtctatggaggcgcaaggttttaagtctgtggttgctgttataggccttccaaacgatccatctgttaggttgcatgaggctttgggatacacagcccggggtacattgcgcgcagctggatacaagcatggtggatggcatgatgttggtttttggcaaagggattttgagttgccagctcctccaaggccagttaggccagttacccagatctga

SEQ ID NO: 61 - DNA, 195 bp, 35S terminator(Cauliflower mosaic virus)
ctgaaatcaccagtctctctctacaaatctatctctctctataataatgtgtgagtagttcccagataagggaattagggttcttatagggtttcgctcatgtgttgagcatataagaaacccttagtatgtatttgtatttgtaaaatacttctatcaataaaatttctaattcctaaaaccaaaatccagtgg

SEQ ID NO: 62 - DNA, 540 bp, The nucleotide sequence of PPO1B(Artificial Sequence)
atgaaagcgttggttctttacagtacaagagatggtcagacccacgccattgcgagctatatcgcaaactgcatgaaggagaagtatgaatgtgacgtcattgatctcttgcacgcgcagcatgtcacccttagccgctacgacaaggtccttgttggggcatcgatacgctatggccatttcaacgccgtgctggacaaatttgttaagcagaatatacaacagctgaactccatgccttctgcattcttcgcggtaaatctgaccgctcgtaagccagaaaaaaggacaccacaaacaaattcatacgtcagaaagttcctcctaggaacgccgtggaagcccgccatgtgcggtgtttttgctggcgccttgcgataccctcggtatcggtgggtggacaaggtgatgatccaattaatcatgaggatgacggggggcgagactgatacttctaaagaagtggagtacactgattgggagcaggtgaaaaaatttgctgaggacttcggaaagctctcctacaagaagacgctgtga

SEQ ID NO: 63 - DNA, 696 bp, The nucleotide sequence of PPO6B(Artificial Sequence)
atgtcaagtcccaacgggaagtaccttatgctgtatagcacgactgatggacacaccaagacaataatggacaccatggcgaagcacattatggaagaggccaaagttcagtgcgacgtcgtagacatgagggacggggacaagtatgaacttgcggcttacgagaaggtcatgctcggcgcctccataaggtacggcttcttcagccgcaccttgcatacatatactacccatcatgttgatgagcttaactccatgccatcggcattctttggtgttaatttaacggcgcggaaaactagcaagaacacagccatgaccaatgcttatacacggaaattcctggatcaatctatgtgggtgccacagctgagtggggtcttcgccggtgcactctggtacccccgctacaacttttttgatcgagtgatgatccagttcatcatgaaggtgacgggcggcgaaacaaatactacaaaagagatcgtctacacggactgggatgcagtgcacaagtttgctactgacttcgtccaactccctgccaccgccattccaagatctaaacctgctacgtcggtgccgccggcgtcagtagcaaactatgataatggtgctcgtgttgcgctggtggtggttggaatttctgcagccatcatcttcggccgcaggctaattttggccaagagattttga

SEQ ID NO: 64 - DNA, 531 bp, The nucleotide sequence of PPO12B(Artificial Sequence)
atgaagaaggcgctgtttttatattcaagtcgtgagggccaaacaaaaaaaatattgaactacattgaaggtgaattgtccaattttgagtgcgagctcgtcgacctccacacgctggacgccattgatttctcggtctatgacagggttttgattggagcaagcatacggtacggccacctaaacaagaaactttatcaattcattgagaataaccgccagcagctggaaaatcataccaaggtggccttcttctgtgtaaatcttactgcaaggaaggaagatcaaggcaaggacacccctgaagggagcgtctacatccagaagttcctgaaaaaatctccctggcagccaaaacttatcggggtgttcgctggcgcgctctactacccgagatatggtttttttgacaagatgatgatcaagctcatcatgacgctgacagatggagagactgatactacaaaggaggtggagtacaccaactggaagaaagtttccctcttcgccaagaagtttgctgagctttga

SEQ ID NO: 65 - protein, 175 aa, The amino acid sequence of PPO-AP(Arsenophonus)
MSYLLLYSGKNGQTKKIILKITEYLRKEGKQCDVRDLNMDKNFNLSVYQKVLVGASIRYGHFNPAVLNFAQNHQKELNTIQSAFFGVNLMARKQGKDTPETNVYVRKFLAKIPWQPTITNVFSGALRYPQYKWLDRIMIQFIMKITGGETNKNKEVEYTDWEKVEYFAREFNALK

SEQ ID NO: 66 - DNA, 528 bp, The nucleotide sequence of PPO-AP(Arsenophonus)
atgagctatttgctactttattctggtaaaaatggtcagactaaaaaaataatacttaaaattactgaatatttacgtaaagaaggtaagcaatgtgatgttagagatttaaatatggataaaaattttaatctttctgtctaccaaaaagtattagtcggtgcatcaatccgttatggtcattttaatcctgcagttttgaattttgcgcaaaatcaccaaaaagagttgaatactatccaaagtgcattttttggcgttaatttaatggccagaaaacagggaaaagatacacctgaaacaaatgtttatgtacgtaaatttttagctaaaattccgtggcaaccaactattactaatgtgttttcgggagcgctacgttatccccaatataaatggttagatcgtattatgatccaatttattatgaaaataacaggcggagaaacgaataaaaataaagaggttgaatatactgattgggaaaaagtcgaatactttgcgcgtgaatttaatgcgcttaaataa

SEQ ID NO: 67 - DNA, 528 bp, The nucleotide sequence of PPO-APA(Artificial Sequence)
atgtcttacctgctgttatattcagggaaaaatggacaaaccaagaagatcattctgaaaataacagagtatcttcgaaaagaaggaaagcaatgtgatgttagagatttgaacatggataagaacttcaacctttctgtatatcagaaggtgctcgttggtgcctcgataagatatggtcatttcaatcccgcagtcctcaattttgctcagaatcaccaaaaggagttaaacactattcaatcagctttctttggcgtgaatttgatggctcgtaaacaaggaaaagatactcctgagacaaatgtgtatgtgaggaagtttcttgccaaaattccatggcaaccaacaatcaccaatgttttcagtggagcgttgaggtatcctcagtacaaatggcttgaccggataatgattcagtttatcatgaagattactggtggtgaaacaaacaaaaacaaggaagttgaatatactgattgggaaaaggtagagtactttgcaagagagtttaatgctttgaaatga

SEQ ID NO: 68 - DNA, 528 bp, The nucleotide sequence of PPO-APB(Artificial Sequence)
atgtcctacctcttgctgtattcggggaaaaatggtcaaaccaagaagatcatcctcaaaataactgaatatcttcgtaaagaaggaaagcagtgcgacgtcagagatcttaacatggacaagaattttaatttaagtgtgtaccagaaggttcttgtcggagcttcaattcgctacggccacttcaaccccgccgtgctgaacttcgcgcagaatcatcaaaaagagctgaacacaattcaatctgccttctttggcgtcaacctgatggcgaggaagcaagggaaggatacaccagaaaccaatgtttatgttcggaagtttttggctaaaattccatggcagccgacgatcaccaacgtatttagcggtgcactcagatatcctcagtacaagtggctggataggataatgatccagttcatcatgaagattactggcggcgagacaaataagaacaaggaggtggagtacacggactgggagaaagtggaatacttcgcccgcgagttcaatgcactaaaatga

SEQ ID NO: 69 - DNA, 25 bp, Primer 1 for detecting the EPSPS gene(Artificial Sequence)
ctggaaggcgaggacgtcatcaata

SEQ ID NO: 70 - DNA, 22 bp, Primer 2 for detecting the EPSPS gene(Artificial Sequence)
tggcggcattgccgaaatcgag

SEQ ID NO: 71 - DNA, 28 bp, Probe 1 for detecting the EPSPS gene(Artificial Sequence)
atgcaggcgatgggcgcccgcatccgta

SEQ ID NO: 72 - DNA, 17 bp, 5'end universal adapter primer 2(Artificial Sequence)
ccaagcggccaagctta

SEQ ID NO: 73 - DNA, 21 bp, 3'end universal adapter primer 2(Artificial Sequence)
tgtttgaacgatcggcgcgcc

SEQ ID NO: 74 - DNA, 1411 bp, Rice actin 1 promoter(Oryza sativa L.)
tactcgaggtcattcatatgcttgagaagagagtcgggatagtccaaaataaaacaaaggtaagattacctggtcaaaagtgaaaacatcagttaaaaggtggtataaagtaaaatatcggtaataaaaggtggcccaaagtgaaatttactcttttctactattataaaaattgaggatgtttttgtcggtactttgatacgtcatttttgtatgaattggtttttaagtttattcgcttttggaaatgcatatctgtatttgagtcgggttttaagttcgtttgcttttgtaaatacagagggatttgtataagaaatatctttagaaaaacccatatgctaatttgacataatttttgagaaaaatatatattcaggcgaattctcacaatgaacaataataagattaaaatagctttcccccgttgcagcgcatgggtattttttctagtaaaaataaaagataaacttagactcaaaacatttacaaaaacaacccctaaagttcctaaagcccaaagtgctatccacgatccatagcaagcccagcccaacccaacccaacccaacccaccccagtccagccaactggacaatagtctccacacccccccactatcaccgtgagttgtccgcacgcaccgcacgtctcgcagccaaaaaaaaaaagaaagaaaaaaaagaaaaagaaaaaacagcaggtgggtccgggtcgtgggggccggaaacgcgaggaggatcgcgagccagcgacgaggccggccctccctccgcttccaaagaaacgccccccatcgccactatatacatacccccccctctcctcccatccccccaaccctaccaccaccaccaccaccacctccacctcctcccccctcgctgccggacgacgagctcctcccccctccccctccgccgccgccgcgccggtaaccaccccgcccctctcctctttctttctccgtttttttttccgtctcggtctcgatctttggccttggtagtttgggtgggcgagaggcggcttcgtgcgcgcccagatcggtgcgcgggaggggcgggatctcgcggctggggctctcgccggcgtggatccggcccggatctcgcggggaatggggctctcggatgtagatctgcgatccgccgttgttgggggagatgatggggggtttaaaatttccgccgtgctaaacaagatcaggaagaggggaaaagggcactatggtttatatttttatatatttctgctgcttcgtcaggcttagatgtgctagatctttctttcttctttttgtgggtagaatttgaatccctcagcattgttcatcggtagtttttcttttcatgatttgtgacaaatgcagcctcgtgcggagcttttttgtaggtagaagtgatcaacc

SEQ ID NO: 75 - DNA, 639 bp, 35S promoter of cauliflower mosaic virus(Artificial Sequence)
ggtccgattgagacttttcaacaaagggtaatatccggaaacctcctcggattccattgcccagctatctgtcactttattgtgaagatagtggaaaaggaaggtggctcctacaaatgccatcattgcgataaaggaaaggccatcgttgaagatgcctctgccgacagtggtcccaaagatggacccccacccacgaggagcatcgtggaaaaagaagacgttccaaccacgtcttcaaagcaagtggattgatgtgatggtccgattgagacttttcaacaaagggtaatatccggaaacctcctcggattccattgcccagctatctgtcactttattgtgaagatagtggaaaaggaaggtggctcctacaaatgccatcattgcgataaaggaaaggccatcgttgaagatgcctctgccgacagtggtcccaaagatggacccccacccacgaggagcatcgtggaaaaagaagacgttccaaccacgtcttcaaagcaagtggattgatgtgatatctccactgacgtaagggatgacgcacaatcccactatccttcgcaagacccttcctctatataaggaagttcatttcatttggagaggacacgctgacaagctgactctagcaga

SEQ ID NO: 76 - DNA, 806 bp, Zea mays heat shock 70 kDa protein intron(Zea mays)
accgtcttcggtacgcgctcactccgccctctgcctttgttactgccacgtttctctgaatgctctcttgtgtggtgattgctgagagtggtttagctggatctagaattacactctgaaatcgtgttctgcctgtgctgattacttgccgtcctttgtagcagcaaaatatagggacatggtagtacgaaacgaagatagaacctacacagcaatacgagaaatgtgtaatttggtgcttagcggtatttatttaagcacatgttggtgttatagggcacttggattcagaagtttgctgttaatttaggcacaggcttcatactacatgggtcaatagtatagggattcatattataggcgatactataataatttgttcgtctgcagagcttattatttgccaaaattagatattcctattctgtttttgtttgtgtgctgttaaattgttaacgcctgaaggaataaatataaatgacgaaattttgatgtttatctctgctcctttattgtgaccataagtcaagatcagatgcacttgttttaaatattgttgtctgaagaaataagtactgacagtattttgatgcattgatctgcttgtttgttgtaacaaaatttaaaaataaagagtttcctttttgttgctctccttacctcctgatggtatctagtatctaccaactgacactatattgcttctctttacatacgtatcttgctcgatgccttctccctagtgttgaccagtgttactcacatagtctttgctcatttcattgtaatgcagataccaagcggcc

SEQ ID NO: 77 - DNA, 1993 bp, Zea mays ubiquitin 1 gene promoter(Zea mays)
ctgcagtgcagcgtgacccggtcgtgcccctctctagagataatgagcattgcatgtctaagttataaaaaattaccacatattttttttgtcacacttgtttgaagtgcagtttatctatctttatacatatatttaaactttactctacgaataatataatctatagtactacaataatatcagtgttttagagaatcatataaatgaacagttagacatggtctaaaggacaattgagtattttgacaacaggactctacagttttatctttttagtgtgcatgtgttctcctttttttttgcaaatagcttcacctatataatacttcatccattttattagtacatccatttagggtttagggttaatggtttttatagactaatttttttagtacatctattttattctattttagcctctaaattaagaaaactaaaactctattttagtttttttatttaataatttagatataaaatagaataaaataaagtgactaaaaattaaacaaataccctttaagaaattaaaaaaactaaggaaacatttttcttgtttcgagtagataatgccagcctgttaaacgccgtcgacgagtctaacggacaccaaccagcgaaccagcagcgtcgcgtcgggccaagcgaagcagacggcacggcatctctgtcgctgcctctggacccctctcgagagttccgctccaccgttggacttgctccgctgtcggcatccagaaattgcgtggcggagcggcagacgtgagccggcacggcaggcggcctcctcctcctctcacggcaccggcagctacgggggattcctttcccaccgctccttcgctttcccttcctcgcccgccgtaataaatagacaccccctccacaccctctttccccaacctcgtgttgttcggagcgcacacacacacaaccagatctcccccaaatccacccgtcggcacctccgcttcaaggtacgccgctcgtcctccccccccccccctctctaccttctctagatcggcgttccggtccatggttagggcccggtagttctacttctgttcatgtttgtgttagatccgtgtttgtgttagatccgtgctgctagcgttcgtacacggatgcgacctgtacgtcagacacgttctgattgctaacttgccagtgtttctctttggggaatcctgggatggctctagccgttccgcagacgggatcgatttcatgattttttttgtttcgttgcatagggtttggtttgcccttttcctttatttcaatatatgccgtgcacttgtttgtcgggtcatcttttcatgcttttttttgtcttggttgtgatgatgtggtctggttgggcggtcgttctagatcggagtagaattctgtttcaaactacctggtggatttattaattttggatctgtatgtgtgtgccatacatattcatagttacgaattgaagatgatggatggaaatatcgatctaggataggtatacatgttgatgcgggttttactgatgcatatacagagatgctttttgttcgcttggttgtgatgatgtggtgtggttgggcggtcgttcattcgttctagatcggagtagaatactgtttcaaactacctggtgtatttattaattttggaactgtatgtgtgtgtcatacatcttcatagttacgagtttaagatggatggaaatatcgatctaggataggtatacatgttgatgtgggttttactgatgcatatacatgatggcatatgcagcatctattcatatgctctaaccttgagtacctatctattataataaacaagtatgttttataattattttgatcttgatatacttggatgatggcatatgcagcagctatatgtggatttttttagccctgccttcatacgctatttatttgcttggtactgtttcttttgtcgatgctcaccctgttgtttggtgttacttctgcag

SEQ ID NO: 78 - DNA, 1176 bp, Phosphomannose isomerase gene(Escherichia coli)
atgcaaaaactcattaactcagtgcaaaactatgcctggggcagcaaaacggcgttgactgaactttatggtatggaaaatccgtccagccagccgatggccgagctgtggatgggcgcacatccgaaaagcagttcacgagtgcagaatgccgccggagatatcgtttcactgcgtgatgtgattgagagtgataaatcgactctgctcggagaggccgttgccaaacgctttggcgaactgcctttcctgttcaaagtattatgcgcagcacagccactctccattcaggttcatccaaacaaacacaattctgaaatcggttttgccaaagaaaatgccgcaggtatcccgatggatgccgccgagcgtaactataaagatcctaaccacaagccggagctggtttttgcgctgacgcctttccttgcgatgaacgcgtttcgtgaattttccgagattgtctccctactccagccggtcgcaggtgcacatccggcgattgctcactttttacaacagcctgatgccgaacgtttaagcgaactgttcgccagcctgttgaatatgcagggtgaagaaaaatcccgcgcgctggcgattttaaaatcggccctcgatagccagcagggtgaaccgtggcaaacgattcgtttaatttctgaattttacccggaagacagcggtctgttctccccgctattgctgaatgtggtgaaattgaaccctggcgaagcgatgttcctgttcgctgaaacaccgcacgcttacctgcaaggcgtggcgctggaagtgatggcaaactccgataacgtgctgcgtgcgggtctgacgcctaaatacattgatattccggaactggttgccaatgtgaaattcgaagccaaaccggctaaccagttgttgacccagccggtgaaacaaggtgcagaactggacttcccgattccagtggatgattttgccttctcgctgcatgaccttagtgataaagaaaccaccattagccagcagagtgccgccattttgttctgcgtcgaaggcgatgcaacgttgtggaaaggttctcagcagttacagcttaaaccgggtgaatcagcgtttattgccgccaacgaatcaccggtgactgtcaaaggccacggccgtttagcgcgtgtttacaacaagctgtaa

SEQ ID NO: 79 - DNA, 29 bp, Primer 3 for detecting the PMI gene sequence(Artificial Sequence)
gctgtaagagcttactgaaaaaattaaca

SEQ ID NO: 80 - DNA, 18 bp, Primer 4 for detecting the PMI gene sequence(Artificial Sequence)
cgatctgcaggtcgacgg

SEQ ID NO: 81 - DNA, 27 bp, Probe 2 for detecting the PMI gene sequence(Artificial Sequence)
tctcttgctaagctgggagctcgatcc